European Patent Application EP 4 286 846 A1, published December 6, 2023. Title: Accurate method for generating a phase diagram of a polymer. Applicant: Max-Planck-Gesellschaft zur Foerderung der Wissenschaften e.V. The sequence listing filed with the application follows.

SEQUENCE LISTING (3 sequences)

SEQ ID NO: 1 - protein, 797 aa, Artificial Sequence
  GFP-tagged Fused in Sarcoma protein purified from BAC construct
MASNDYTQQATQSYGAYPTQPGQGYSQQSSQPYGQQSYSGYSQSTDTSGYGQSSYSSYGQSQNTGYGTQSTPQGYGSTGGYGSSQSSQSSYGQQSSYPGYGQQPAPSSTSGSYGSSSQSSSYGQPQSGSYSQQPSYGGQQQSYGQQQSYNPPQGYGQQNQYNSSSGGGGGGGGGGNYGQDQSSMSSGGGSGGGYGNQDQSGGGGSGGYGQQDRGGRGRGGSGGGGGGGGGGYNRSSGGYEPRGRGGGRGGRGGMGGSDRGGFNKFGGPRDQGSRHDSEQDNSDNNTIFVQGLGENVTIESVADYFKQIGIIKTNKKTGQPMINLYTDRETGKLKGEATVSFDDPPSAKAAIDWFDGKEFSGNPIKVSFATRRADFNRGGGNGRGGRGRGGPMGRGGYGGGGSGGGGRGGFPSGGGGGGGQQRAGDWKCPNPTCENMNFSWRNECNQCKAPKPDGPGGGPGGSHMGGNYGDDRRGGRGGYDRGGYRGRGGDRGGFRGGRGGGDRGGFGPGKMDSRGEHRQDRRERPYGAPGSAGSAAGSGMVSKGEELFTGVVPILVELDGDVNGHKFSVSGEGEGDATYGKLTLKFICTTGKLPVPWPTLVTTLTYGVQCFSRYPDHMKQHDFFKSAMPEGYVQERTIFFKDDGNYKTRAEVKFEGDTLVNRIELKGIDFKEDGNILGHKLEYNYNSHNVYIMADKQKNGIKVNFKIRHNIEDGSVQLADHYQQNTPIGDGPVLLPDNHYLSTQSKLSKDPNEKRDHMVLLEFVTAAGITLGMDELYKLEVLFQGPGSSHHHHHHSG

SEQ ID NO: 2 - protein, 953 aa, Artificial Sequence
  PGL-3-6xHis-mEGFP protein purified in SF9 insect cells from baculovirus construct
MEANKRQIVEVDGIKSYFFPHLAHYLASNDELLVNNIAQANKLAAFVLGATDKRPSNEEIAEMILPNDSSAYVLAAGMDVCLILGDDFRPKFDSGAEKLSQLGQAHDLAPIIDDEKKISMLARKTKLKKSNDAKILQVLLKVLGAEEAEEKFVELSELSSALDLDFDVYVLAKLLGFASEELQEEIEIIRDNVTDAFEACKPLLKKLMIEGPKIDSVDPFTQLLLTPQEESIEKAVSHIVARFEEASAVEDDESLVLKSQLGYQLIFLVVRSLADGKRDASRTIQSLMPSSVRAEVFPGLQRSVFKSAVFLASHIIQVFLGSMKSFEDWAFVGLAEDLESTWRRRAIAELLKKFRISVLEQCFSQPIPLLPQSELNNETVIENVNNALQFALWITEFYGSESEKKSLNQLQFLSPKSKNLLVDSFKKFAQGLDSKDHVNRIIESLEKSSSSEPSATAKQTTTSNGPTTVSTAAQVVTVEKMPFSRQTIPCEGTDLANVLNSAKIIGESVTVAAHDVIPEKLNAEKNDNTPSTASPVQFSSDGWDSPTKSVALPPKISTLEEEQEEDTTITKVSPQPQERTGTAWGSGDATPVPLATPVNEYKVSGFGAAPVASGFGQFASSNGTSGRGSYGGGRGGDRGGRGAYGGDRGRGGSGDGSRGYRGGDRGGRGSYGEGSRGYQGGRAGFFGGSRGGSSRENLYFQSSAHHHHHHHVMVSKGEELFTGVVPILVELDGDVNGHKFSVSGEGEGDATYGKLTLKFICTTGKLPVPWPTLVTTLTYGVQCFSRYPDHMKQHDFFKSAMPEGYVQERTIFFKDDGNYKTRAEVKFEGDTLVNRIELKGIDFKEDGNILGHKLEYNYNSHNVYIMADKQKNGIKVNFKIRHNIEDGSVQLADHYQQNTPIGDGPVLLPDNHYLSTQSALSKDPNEKRDHMVLKEFVTAAGITLGMDELYKGA

SEQ ID NO: 3 - RNA, 250 nt, Artificial Sequence
  Poly(A) RNA
aaaaaaaaaaaaaaaaaaaaaaaaaaaaaaaaaaaaaaaaaaaaaaaaaaaaaaaaaaaaaaaaaaaaaaaaaaaaaaaaaaaaaaaaaaaaaaaaaaaaaaaaaaaaaaaaaaaaaaaaaaaaaaaaaaaaaaaaaaaaaaaaaaaaaaaaaaaaaaaaaaaaaaaaaaaaaaaaaaaaaaaaaaaaaaaaaaaaaaaaaaaaaaaaaaaaaaaaaaaaaaaaaaaaaaaaaaaaaaaaaaaaaaaaaa